European Patent Specification EP 4 056 695 B1, published October 18, 2023. Title: Novel ATP phosphoribosyltransferase variant and a method for producing L-valine using the same. Applicant: CJ CheilJedang Corporation. The sequence listing filed with the application follows.

SEQUENCE LISTING (11 sequences)

SEQ ID NO: 1 - protein, 281 aa, Artificial Sequence
  ATP phosphoribosyl-transferase variant
MLKIAVPNKGSLSERAMEILTEAGYAGRGDSKSLNVFDEANNVEFFFLRPKDIAIYVAGGQLDLGITGRDLARDSQADVHEVLSLGFGSSTFRYAAPADEEWSIEKLDGKRIATSYPNLVRDDLAARGLFAEVLRLDGAVEVSIKLGVADAIADVVSTGRTLRQQGLAPFGEVLCTSEAVIVGRKDEKVTPEQQILLRRIQGILHAQNFLMLDYNVDRDNLDAATAVTPGLSGPTVSPLARDNWVAVRAMVPRRSANAIMDKLAGLGAEAILASEIRIARI

SEQ ID NO: 2 - DNA, 846 bp, Artificial Sequence
  ATP phosphoribosyl-transferase variant coding gene
atgttgaaaatcgctgtcccaaacaagggctcgctgtccgagcgcgccatggaaatcctcaccgaagcaggctacgcaggccgtggagattccaaatccctcaacgtttttgatgaagcaaacaacgttgaattcttcttccttcgccctaaagatatcgccatctacgttgctggtggccagctcgatttgggtatcaccggccgcgaccttgctcgcgattcccaggctgatgtccacgaagttctttccctcggcttcggttcctccactttccgttacgcagcaccagctgatgaagagtggagcatcgaaaagctcgacggcaagcgcatcgctacctcttaccccaaccttgttcgcgatgacctcgcagcacgtgggcttttcgctgaggtgctccgcctcgacggtgcagtagaggtatccatcaagcttggtgtcgcagatgccatcgccgatgttgtatccaccggccgcacgctgcgtcagcaaggtcttgcacctttcggcgaggttctgtgtacctctgaggctgtcattgttggccgcaaggatgaaaaggtcaccccagagcagcagatcctgcttcgccgcatccagggaattttgcacgcgcagaacttcctcatgctggattacaacgtcgaccgcgacaacctggacgctgccactgcagtaaccccaggcctatccggcccaacggtatccccactggcacgcgacaactgggttgctgtacgcgccatggtgccacgcaggtcagctaacgccatcatggataagcttgctggactcggcgctgaagccatcctggcttctgaaatccgcatcgcccgcatctag

SEQ ID NO: 3 - protein, 281 aa, Artificial Sequence
  Wild-type ATP phosphoribosyl-transferase
MLKIAVPNKGSLSERAMEILTEAGYAGRGDSKSLNVFDEANNVEFFFLRPKDIAIYVAGGQLDLGITGRDLARDSQADVHEVLSLGFGSSTFRYAAPADEEWSIEKLDGKRIATSYPNLVRDDLAARGLSAEVLRLDGAVEVSIKLGVADAIADVVSTGRTLRQQGLAPFGEVLCTSEAVIVGRKDEKVTPEQQILLRRIQGILHAQNFLMLDYNVDRDNLDAATAVTPGLSGPTVSPLARDNWVAVRAMVPRRSANAIMDKLAGLGAEAILASEIRIARI

SEQ ID NO: 4 - DNA, 846 bp, Artificial Sequence
  Wild-type ATP phosphoribosyl-transferase coding gene
atgttgaaaatcgctgtcccaaacaagggctcgctgtccgagcgcgccatggaaatcctcaccgaagcaggctacgcaggccgtggagattccaaatccctcaacgtttttgatgaagcaaacaacgttgaattcttcttccttcgccctaaagatatcgccatctacgttgctggtggccagctcgatttgggtatcaccggccgcgaccttgctcgcgattcccaggctgatgtccacgaagttctttccctcggcttcggttcctccactttccgttacgcagcaccagctgatgaagagtggagcatcgaaaagctcgacggcaagcgcatcgctacctcttaccccaaccttgttcgcgatgacctcgcagcacgtgggctttccgctgaggtgctccgcctcgacggtgcagtagaggtatccatcaagcttggtgtcgcagatgccatcgccgatgttgtatccaccggccgcacgctgcgtcagcaaggtcttgcacctttcggcgaggttctgtgtacctctgaggctgtcattgttggccgcaaggatgaaaaggtcaccccagagcagcagatcctgcttcgccgcatccagggaattttgcacgcgcagaacttcctcatgctggattacaacgtcgaccgcgacaacctggacgctgccactgcagtaaccccaggcctatccggcccaacggtatccccactggcacgcgacaactgggttgctgtacgcgccatggtgccacgcaggtcagctaacgccatcatggataagcttgctggactcggcgctgaagccatcctggcttctgaaatccgcatcgcccgcatctag

SEQ ID NO: 5 - DNA, 36 bp, Artificial Sequence
  hisG_1F
tcgagctcggtacccatgttgaaaatcgctgtccca

SEQ ID NO: 6 - DNA, 44 bp, Artificial Sequence
  hisG_2R
gtcgaggcggagcacctcagcgaaaagcccacgtgctgcgaggt

SEQ ID NO: 7 - DNA, 44 bp, Artificial Sequence
  hisG_3F
acctcgcagcacgtgggcttttcgctgaggtgctccgcctcgac

SEQ ID NO: 8 - DNA, 36 bp, Artificial Sequence
  hisG_4R
ctctagaggatccccctagatgcgggcgatgcggat

SEQ ID NO: 9 - DNA, 21 bp, Artificial Sequence
  hisG_5F
atgttgaaaatcgctgtccca

SEQ ID NO: 10 - DNA, 21 bp, Artificial Sequence
  hisG_6R
ctagatgcgggcgatgcggat

SEQ ID NO: 11 - DNA, 5803 bp, Artificial Sequence
  pDCM2
gttcgcttgctgtccataaaaccgcccagtctagctatcgccatgtaagcccactgcaagctacctgctttctctttgcgcttgcgttttcccttgtccagatagcccagtagctgacattcatccggggtcagcaccgtttctgcggactggctttctacgtgttccgcttcctttagcagcccttgcgccctgagtgcttgcggcagcgtgaagctagcttttatcgccattcgccattcaggctgcgcaactgttgggaagggcgatcggtgcgggcctcttcgctattacgccagctggcgaaagggggatgtgctgcaaggcgattaagttgggtaacgccagggttttcccagtcacgacgttgtaaaacgacggccagtgaattcgagctcggtacccggggatcctctagagtcgacctgcaggcatgcaagcttggcgtaatcatggtcatagctgtttcctgtgtgaaattgttatccgctcacaattccacacaacatacgagccggaagcataaagtgtaaagcctggggtgcctaatgagtgagctaactcacattaattgcgttgcgctcactgcccgctttccagtcgggaaacctgtcgtgccagctgcattaatgaatcggccaacgcgcggggagaggcggtttgcgtattgggcgctcttccgcttcctcgctcactgactcgctgcgctcggtcgttcggctgcggcgagcggtatcagctcactcaaaggcggtaatacggttatccacagaatcaggggataacgcaggaaagaacatgtgagcaaaaggccagcaaaaggccaggaaccgtaaaaaggccgcgttgctggcgtttttccataggctccgcccccctgacgagcatcacaaaaatcgacgctcaagtcagaggtggcgaaacccgacaggactataaagataccaggcgtttccccctggaagctccctcgtgcgctctcctgttccgaccctgccgcttaccggatacctgtccgcctttctcccttcgggaagcgtggcgctttctcaatgctcacgctgtaggtatctcagttcggtgtaggtcgttcgctccaagctgggctgtgtgcacgaaccccccgttcagcccgaccgctgcgccttatccggtaactatcgtcttgagtccaacccggtaagacacgacttatcgccactggcagcagccactggtaacaggattagcagagcgaggtatgtaggcggtgctacagagttcttgaagtggtggcctaactacggctacactagaaggacagtatttggtatctgcgctctgctgaagccagttaccttcggaaaaagagttggtagctcttgatccggcaaacaaaccaccgctggtagcggtggtttttttgtttgcaagcagcagattacgcgcagaaaaaaaggatctcaagaagatcctttgatcttttctacggggtctgacgctcagtggaacgaaaactcacgttaagggattttggtcatgagattatcaaaaaggatcttcacctagatccttttggggtgggcgaagaactccagcatgagatccccgcgctggaggatcatccagccctgatagaaacagaagccactggagcacctcaaaaacaccatcatacactaaatcagtaagttggcagcatcacccgacgcactttgcgccgaataaatacctgtgacggaagatcacttcgcagaataaataaatcctggtgtccctgttgataccgggaagccctgggccaacttttggcgaaaatgagacgttgatcggcacgtaagaggttccaactttcaccataatgaaataagatcactaccgggcgtattttttgagttatcgagattttcaggagctgatagaaacagaagccactggagcacctcaaaaacaccatcatacactaaatcagtaagttggcagcatcacccgacgcactttgcgccgaataaatacctgtgacggaagatcacttcgcagaataaataaatcctggtgtccctgttgataccgggaagccctgggccaacttttggcgaaaatgagacgttgatcggcacgtaagaggttccaactttcaccataatgaaataagatcactaccgggcgtattttttgagttatcgagattttcaggagctctttggcatcgtctctcgcctgtcccctcagttcagtaatttcctgcatttgcctgtttccagtcggtagatattccacaaaacagcagggaagcagcgcttttccgctgcataaccctgcttcggggtcattatagcgattttttcggtatatccatcctttttcgcacgatatacaggattttgccaaagggttcgtgtagactttccttggtgtatccaacggcgtcagccgggcaggataggtgaagtaggcccacccgcgagcgggtgttccttcttcactgtcccttattcgcacctggcggtgctcaacgggaatcctgctctgcgaggctggccggctaccgccggcgtaacagatgagggcaagcggatggctgatgaaaccaagccaaccaggaagggcagcccacctatcaaggtgtactgccttccagacgaacgaagagcgattgaggaaaaggcggcggcggccggcatgagcctgtcggcctacctgctggccgtcggccagggctacaaaatcacgggcgtcgtggactatgagcacgtccgcgagggcgtcccggaaaacgattccgaagcccaacctttcatagaaggcggcggtggaatcgaaatctcgtgatggcaggttgggcgtcgcttggtcggtcatttcgaaaaaggttaggaatacggttagccatttgcctgcttttatatagttcantatgggattcacctttatgttgataagaaataaaagaaaatgccaataggatatcggcattttcttttgcgtttttatttgttaactgttaattgtccttgttcaaggatgctgtctttgacaacagatgttttcttgcctttgatgttcagcaggaagctcggcgcaaacgttgattgtttgtctgcgtagaatcctctgtttgtcatatagcttgtaatcacgacattgtttcctttcgcttgaggtacagcgaagtgtgagtaagtaaaggttacatcgttaggcggatcaagatccatttttaacacaaggccagttttgttcagcggcttgtatgggccagttaaagaattagaaacataaccaagcatgtaaatatcgttagacgtaatgccgtcaatcgtcatttttgatccgcgggagtcagtgaacaggtaccatttgccgttcattttaaagacgttcgcgcgttcaatttcatctgttactgtgttagatgcaatcagcggtttcatcacttttttcagtgtgtaatcatcgtttagctcaatcataccgagagcgccgtttgctaactcagccgtgcgttttttatcgctttgcagaagtttttgactttcttgacggaagaatgatgtgcttttgccatagtatgctttgttaaataaagattcttcgccttggtagccatcttcagttccagtgtttgcttcaaatactaagtatttgtggcctttatcttctacgtagtgaggatctctcagcgtatggttgtcgcctgagctgtagttgccttcatcgatgaactgctgtacattttgatacgtttttccgtcaccgtcaaagattgatttataatcctctacaccgttgatgttcaaagagctgtctgatgctgatacgttaacttgtgcagttgtcagtgtttgtttgccgtaatgtttaccggagaaatcagtgtagaataaacggatttttccgtcagatgtaaatgtggctgaacctgaccattcttgtgtttggtcttttaggatagaatcatttgcatcgaatttgtcgctgtctttaaagacgcggccagcgtttttccagctgtcaatagaagtttcgccgactttttgatagaacatgtaaatcgatgtgtcatccgcatttttaggatctccggctaatgcaaagacgatgtggtagccgtgatagtttgcgacagtgccgtcagcgttttgtaatggccagctgtcccaaacgtccaggccttttgcagaagagatatttttaattgtggacgaatcaaattcagaaacttgatatttttcatttttttgctgttcagggatttgcagcatatcatggcgtgtaatatgggaaatgccgtatgtttccttatatggcttttggttcgtttctttcgcaaacgcttgagttgcgcctcctgccagcagtgcggtagtaaaggttaatactgttgcttgttttgcaaactttttgatgttcatcgttcatgtctccttttttatgtactgtgttagcggtctgcttcttccagccctcctgtttgaagatggcaagttagttacgcacaataaaaaaagacctaaaatatgtaaggggtgacgccaaagtatacactttgccctttacacattttaggtcttgcctgctttatcagtaacaaacccgcgcgatttacttttcgacctcattctattagactctcgtttggattgcaactggtctattttcctcttttgtttgatagaaaatcataaaaggatttgcagactacgggcctaaagaactaaaaaatctatctgtttcttttcattctctgtattttttatagtttctgttgcatgggcataaagttgcctttttaatcacaattcagaaaatatcataatatctcatttcactaaataatagtgaacggcaggtatatgtgatgggttaaaaaggatcaccccagagtcccgctcagaagaactcgtcaagaaggcgatagaaggcgatgcgctgcgaatcgggagcggcgataccgtaaagcacgaggaagcggtcagcccattcgccgccaagctcttcagcaatatcacgggtagccaacgctatgtcctgatagcggtccgccacacccagccggccacagtcgatgaatccagaaaagcggccattttccaccatgatattcggcaagcaggcatcgccatgggtcacgacgagatcctcgccgtcgggcatccgcgccttgagcctggcgaacagttcggctggcgcgagcccctgatgctcttcgtccagatcatcctgatcgacaagaccggcttccatccgagtacgtgctcgctcgatgcgatgtttcgcttggtggtcgaatgggcaggtagccggatcaagcgtatgcagccgccgcattgcatcagccatgatggatactttctcggcaggagcaaggtgagatgacaggagatcctgccccggcacttcgcccaatagcagccagtcccttcccgcttcagtgacaacgtcgagacagctgcgcaaggaacgcccgtcgtggccagccacgatagccgcgctgcctcgtcttggagttcattcagggcaccggacaggtcggtcttgacaaaaagaaccgggcgcccctgcgctgacagccggaacacggcggcatcagagcagccgattgtctgttgtgcccagtcatagccgaatagcctctccacccaagcggccggagaacctgcgtgcaatccatcttgttcaatcatgcgaaacgatcctcatcctgtctcttgatcagatcttgatcccctgcgccatcagatccttggcggcaagaaagccatccagtttactttgcagggcttcccaaccttaccagagggcgccccagctggcaattccg